European Patent Application EP 4 450 075 A1, published October 23, 2024. Title: TREATMENT OF HEPATOPATHY USING ADIPOSE-DERIVED MESENCHYMAL STEM CELL LINE. Applicant: 慶應義塾. The sequence listing filed with the application follows.

SEQUENCE LISTING (10 sequences)

SEQ ID NO: 1 - DNA, 20 bp, synthetic construct
  source 1..20: mol_type = other DNA
cgttaccttggtaaccggct

SEQ ID NO: 2 - DNA, 20 bp, synthetic construct
  source 1..20: mol_type = other DNA
agccctgtattccgtctcct

SEQ ID NO: 3 - DNA, 20 bp, synthetic construct
  source 1..20: mol_type = other DNA
gaaggaccagctggacaaca

SEQ ID NO: 4 - DNA, 15 bp, synthetic construct
  source 1..15: mol_type = other DNA
tcagcttctctccca

SEQ ID NO: 5 - DNA, 20 bp, synthetic construct
  source 1..20: mol_type = other DNA
cgctttaccttcatccgctc

SEQ ID NO: 6 - DNA, 20 bp, synthetic construct
  source 1..20: mol_type = other DNA
gggctcttttggtgtgttgg

SEQ ID NO: 7 - DNA, 20 bp, synthetic construct
  source 1..20: mol_type = other DNA
agagacttccagccagttgc

SEQ ID NO: 8 - DNA, 20 bp, synthetic construct
  source 1..20: mol_type = other DNA
tctgacagtgcatcatcgct

SEQ ID NO: 9 - DNA, 20 bp, synthetic construct
  source 1..20: mol_type = other DNA
gaaggtcggtgtgaacggat

SEQ ID NO: 10 - DNA, 20 bp, synthetic construct
  source 1..20: mol_type = other DNA
accagcttcccattctcagc